European Patent Application EP 4 796 181 A1, published August 26, 2026. Title: NEUTRALIZING ANTIBODIES AGAINST GLYCOPROTEIN 130, METHODS AND USES THEREOF. Applicant: FUNDACIÓ PRIVADA INSTITUT D'INVESTIGACIÓ ONCOLÒGICA DE VALL HEBRON. Application EP. The sequence listing filed with the application follows.

SEQUENCE LISTING (39 sequences)

SEQ ID NO: 1 - protein, 8 aa, synthetic construct
GFTFTNYW

SEQ ID NO: 2 - protein, 8 aa, synthetic construct
INVAGDNI

SEQ ID NO: 3 - protein, 11 aa, synthetic construct
AKDPGGPPFDY

SEQ ID NO: 4 - protein, 6 aa, synthetic construct
QTIYNS

SEQ ID NO: 5 - skipped

SEQ ID NO: 6 - protein, 8 aa, synthetic construct
HQYYSWYT

SEQ ID NO: 7 - protein, 25 aa, synthetic construct
AVQLVETGGGLVYPGRSLKLSCVGS

SEQ ID NO: 8 - protein, 17 aa, synthetic construct
MYWIRQAPGKGLEWVAS

SEQ ID NO: 9 - protein, 38 aa, synthetic construct
NYSDSVKGRFSISRDNAANTVYLQMNSLRSEDTATYYC

SEQ ID NO: 10 - protein, 11 aa, synthetic construct
WGQGVMVTVSS

SEQ ID NO: 11 - protein, 26 aa, synthetic construct
DIQMTQSPSLLSASVGDRVTLTCKAS

SEQ ID NO: 12 - protein, 17 aa, synthetic construct
LAWYQQKLGEAPKLLIY

SEQ ID NO: 13 - protein, 36 aa, synthetic construct
SLQTGIPSRFSGSGFGTDFTLTISSLQPEDVAAYFC

SEQ ID NO: 14 - protein, 10 aa, synthetic construct
FGAGTKLELK

SEQ ID NO: 15 - protein, 118 aa, synthetic construct
AVQLVETGGGLVYPGRSLKLSCVGSGFTFTNYWMYWIRQAPGKGLEWVASINVAGDNINYSDSVKGRFSISRDNAANTVYLQMNSLRSEDTATYYCAKDPGGPPFDYWGQGVMVTVSS

SEQ ID NO: 16 - protein, 106 aa, synthetic construct
DIQMTQSPSLLSASVGDRVTLTCKASQTIYNSLAWYQQKLGEAPKLLIYSANSLQTGIPSRFSGSGFGTDFTLTISSLQPEDVAAYFCHQYYSWYTFGAGTKLELK

SEQ ID NO: 17 - protein, 16 aa, synthetic construct
TGSTSGSGKPGSGEGS

SEQ ID NO: 18 - protein, 5 aa, synthetic construct
GSGGS

SEQ ID NO: 19 - protein, 4 aa, synthetic construct
GGGS

SEQ ID NO: 20 - protein, 4 aa, synthetic construct
GGSG

SEQ ID NO: 21 - protein, 5 aa, synthetic construct
GGSGG

SEQ ID NO: 22 - protein, 5 aa, synthetic construct
GSGSG

SEQ ID NO: 23 - protein, 5 aa, synthetic construct
GSGGG

SEQ ID NO: 24 - protein, 5 aa, synthetic construct
GGGSG

SEQ ID NO: 25 - protein, 5 aa, synthetic construct
GSSSG

SEQ ID NO: 26 - protein, 22 aa, synthetic construct
VKQTLNFDLLKLAGDVESNPGP

SEQ ID NO: 27 - protein, 20 aa, synthetic construct
QCTNYALLKLAGDVESNPGP

SEQ ID NO: 28 - protein, 19 aa, synthetic construct
ATNFSLLKQAGDVEENPGP

SEQ ID NO: 29 - protein, 18 aa, synthetic construct
EGRGSLLTCGDVEENPGP

SEQ ID NO: 30 - protein, 63 aa, synthetic construct
GSGSRVTELLYRMKRAETYCPRPLLAIHPTEARHKQKIVAPVKQLLNFDLLKLAGDVESNPGP

SEQ ID NO: 31 - protein, 19 aa, synthetic construct
LLCFLLLLLSGDVELNPGP

SEQ ID NO: 32 - protein, 20 aa, synthetic construct
HHFMFLLLLLAGDIELNPGP

SEQ ID NO: 33 - protein, 20 aa, synthetic construct
WFLVLLSFILSGDIEVNPGP

SEQ ID NO: 34 - protein, 20 aa, synthetic construct
KNCAMYMLLLSGDVETNPGP

SEQ ID NO: 35 - protein, 20 aa, synthetic construct
MVISQLMLKLAGDVEENPGP

SEQ ID NO: 36 - protein, 22 aa, synthetic construct
GSGATNFSLLKQAGDVEENPGP

SEQ ID NO: 37 - protein, 21 aa, synthetic construct
GSGEGRGSLLTCGDVEENPGP

SEQ ID NO: 38 - protein, 23 aa, synthetic construct
GSGQCTNYALLKLAGDVESNPGP

SEQ ID NO: 39 - protein, 8 aa, synthetic construct
  SITE 2: note = Xaa can be any naturally occurring amino acid
  SITE 4: note = Xaa can be any naturally occurring amino acid
DXEXNPGP